European Patent Specification EP 4 153 194 B1, published February 18, 2026. Title: METHODS FOR ENHANCING ADOPTIVE CELL TRANSFER IMMUNOTHERAPIES. Applicant: HANSA BIOPHARMA AB. The sequence listing filed with the application follows.

SEQUENCE LISTING (90 sequences)

SEQ ID NO: 1 - protein, 339 aa, Streptococcus pyogenes
MRKRCYSTSAAVLAAVTLFVLSVDRGVIADSFSANQEIRYSEVTPYHVTSVWTKGVTPPANFTQGEDVFHAPYVANQGWYDITKTFNGKDDLLCGAATAGNMLHWWFDQNKDQIKRYLEEHPEKQKINFNGEQMFDVKEAIDTKNHQLDSKLFEYFKEKAFPYLSTKHLGVFPDHVIDMFINGYRLSLTNHGPTPVKEGSKDPRGGIFDAVFTRGDQSKLLTSRHDFKEKNLKEISDLIKKELTEGKALGLSHTYANVRINHVINLWGADFDSNGNLKAIYVTDSDSNASIGMKKYFVGVNSAGKVAISAKEIKEDNIGAQVLGLFTLSTGQDSWNQTN

SEQ ID NO: 2 - protein, 310 aa, Streptococcus pyogenes
DSFSANQEIRYSEVTPYHVTSVWTKGVTPPANFTQGEDVFHAPYVANQGWYDITKTFNGKDDLLCGAATAGNMLHWWFDQNKDQIKRYLEEHPEKQKINFNGEQMFDVKEAIDTKNHQLDSKLFEYFKEKAFPYLSTKHLGVFPDHVIDMFINGYRLSLTNHGPTPVKEGSKDPRGGIFDAVFTRGDQSKLLTSRHDFKEKNLKEISDLIKKELTEGKALGLSHTYANVRINHVINLWGADFDSNGNLKAIYVTDSDSNASIGMKKYFVGVNSAGKVAISAKEIKEDNIGAQVLGLFTLSTGQDSWNQTN

SEQ ID NO: 3 - protein, 349 aa, Streptococcus pyogenes
MKTIAYPNKPHSLSAGLLTAIAIFSLASSNITYADDYQRNATEAYAKEVPHQITSVWTKGVTPLTPEQFRYNNEDVIHAPYLAHQGWYDITKAFDGKDNLLCGAATAGNMLHWWFDQNKTEIEAYLSKHPEKQKIIFNNQELFDLKAAIDTKDSQTNSQLFNYFRDKAFPNLSARQLGVMPDLVLDMFINGYYLNVFKTQSTDVNRPYQDKDKRGGIFDAVFTRGDQTTLLTARHDLKNKGLNDISTIIKQELTEGRALALSHTYANVSISHVINLWGADFNAEGNLEAIYVTDSDANASIGMKKYFVGINAHGHVAISAKKIEGENIGAQVLGLFTLSSGKDIWQKLS

SEQ ID NO: 4 - protein, 315 aa, Streptococcus pyogenes
DDYQRNATEAYAKEVPHQITSVWTKGVTPLTPEQFRYNNEDVIHAPYLAHQGWYDITKAFDGKDNLLCGAATAGNMLHWWFDQNKTEIEAYLSKHPEKQKIIFNNQELFDLKAAIDTKDSQTNSQLFNYFRDKAFPNLSARQLGVMPDLVLDMFINGYYLNVFKTQSTDVNRPYQDKDKRGGIFDAVFTRGDQTTLLTARHDLKNKGLNDISTIIKQELTEGRALALSHTYANVSISHVINLWGADFNAEGNLEAIYVTDSDANASIGMKKYFVGINAHGHVAISAKKIEGENIGAQVLGLFTLSSGKDIWQKLS

SEQ ID NO: 5 - protein, 313 aa, Streptococcus pyogenes
DDYQRNATEAYAKEVPHQITSVWTKGVTPLTPEQFRYNNEDVFHAPYVANQGWYDITKAFDGKDNLLCGAATAGNMLHWWFDQNKDQIKRYLEEHPEKQKINFNGDNMFDVKKAIDTKNHQLDSKLFNYFKEKAFPGLSARRIGVFPDHVIDMFINGYRLSLTNHGPTPVKEGSKDPRGGIFDAVFTRGNQSKLLTSRHDFKNKNLNDISTIIKQELTKGKALGLSHTYANVSINHVINLWGADFNAEGNLEAIYVTDSDSNASIGMKKYFVGVNAHGHVAISAKKIEGENIGAQVLGLFTLSTGQDSWQKLS

SEQ ID NO: 6 - protein, 315 aa, Streptococcus pyogenes
DDYQRNATEAYAKEVPHQITSVWTKGVTPLTPEQFRYNNEDVIHAPYLANQGWYDITKAFDGKDNLLCGAATAGNMLHWWFDQNKTEIEAYLSKHPEKQKIIFRNQELFDLKEAIRTKDSQTNSQLFEYFRDKAFPYLSARQLGVMPDLVLDMFINGYYLNVFKTQSTDVKRPYQDKDKRGGIFDAVFTRGNQTTLLTARHDLKNKGLNDISTIIKEELTKGRALALSHTYANVSISHVINLWGADFNAEGNLEAIYVTDSDANASIGMKKYFVGINKHGHVAISAKKIEGENIGAQVLGLFTLSSGKDIWQKLN

SEQ ID NO: 7 - protein, 315 aa, Streptococcus pyogenes
DDYQRNATEAYAKEVPHQITSVWTKGVTPLTPEQFRYNNEDVIHAPYLAHQGWYDITKTFNGKDNLLCGAATAGNMLHWWFDQNKTEIEAYLSKHPEKQKIIFNNEELFDLKAAIDTKDSQTNSQLFNYFKEKAFPNLSTRQLGVMPDLVLDMFINGYYLNVFKTQSTDVNRPYQDKDKRGGIFDAVFTRGNQTTLLTARHDFKEKGLKDISTIIKQELTEGRALALSHTYANVSISHVINLWGADFDAEGNLKAIYVTDSDANASIGMKKYFVGINAHGKVAISAKKIEGENIGAQVLGLFTLSSGKDIWQQLS

SEQ ID NO: 8 - protein, 315 aa, Streptococcus pyogenes
DSFSANQEIRYSEVTPYHVTSVWTKGVTPLTPEQFRYNNEDVIHAPYLAHQGWYDITKAFDGKDNLLCGAATAGNMLHWWFDQNKTEIEAYLSKHPEKQKIIFNNQELFDLKAAIDTKDSQTNSQLFNYFRDKAFPNLSARQLGVMPDLVLDMFINGYYLNVFKTQSTDVNRPYQDKDKRGGIFDAVFTRGDQTTLLTARHDLKNKGLNDISTIIKQELTEGRALALSHTYANVSISHVINLWGADFNAEGNLEAIYVTDSDANASIGMKKYFVGINAHGHVAISAKKIEGENIGAQVLGLFTLSSGKDIWQKLS

SEQ ID NO: 9 - protein, 295 aa, Streptococcus pyogenes
SVWTKGVTPLTPEQFRYNNEDVIHAPYLAHQGWYDITKAFDGKDNLLCGAATAGNMLHWWFDQNKTEIEAYLSKHPEKQKIIFNNQELFDLKAAIDTKDSQTNSQLFNYFRDKAFPNLSARQLGVMPDLVLDMFINGYYLNVFKTQSTDVNRPYQDKDKRGGIFDAVFTRGDQTTLLTARHDLKNKGLNDISTIIKQELTEGRALALSHTYANVSISHVINLWGADFNAEGNLEAIYVTDSDANASIGMKKYFVGINAHGHVAISAKKIEGENIGAQVLGLFTLSSGKDIWQKLS

SEQ ID NO: 10 - protein, 314 aa, Streptococcus pyogenes
DDYQRNATEAYAKEVPHQITSVWTKGVTPLTPEQFTQGEDVIHAPYLAHQGWYDITKAFDGKDNLLCGAATAGNMLHWWFDQNKTEIEAYLSKHPEKQKIIFNNQELFDLKAAIDTKDSQTNSQLFNYFRDKAFPNLSARQLGVMPDLVLDMFINGYYLNVFKTQSTDVNRPYQDKDKRGGIFDAVFTRGDQTTLLTARHDLKNKGLNDISTIIKQELTEGRALALSHTYANVSISHVINLWGADFNAEGNLEAIYVTDSDANASIGMKKYFVGINAHGHVAISAKKIEGENIGAQVLGLFTLSSGKDIWQKLS

SEQ ID NO: 11 - protein, 312 aa, Streptococcus pyogenes
DDYQRNATEAYAKEVPHQITSVWTKGVTPPEQFTQGEDVIHAPYLAHQGWYDITKAFDGKDNLLCGAATAGNMLHWWFDQNKTEIEAYLSKHPEKQKIIFNNQELFDLKAAIDTKDSQTNSQLFNYFRDKAFPNLSARQLGVMPDLVLDMFINGYYLNVFKTQSTDVNRPYQDKDKRGGIFDAVFTRGDQTTLLTARHDLKNKGLNDISTIIKQELTEGRALALSHTYANVSISHVINLWGADFNAEGNLEAIYVTDSDANASIGMKKYFVGINAHGHVAISAKKIEGENIGAQVLGLFTLSSGKDIWQKLS

SEQ ID NO: 12 - protein, 313 aa, Streptococcus pyogenes
DDYQRNATEAYAKEVPHQITSVWTKGVTPPEQFRYNNEDVIHAPYLAHQGWYDITKAFDGKDNLLCGAATAGNMLHWWFDQNKTEIEAYLSKHPEKQKIIFNNQELFDLKAAIDTKDSQTNSQLFNYFRDKAFPNLSARQLGVMPDLVLDMFINGYYLNVFKTQSTDVNRPYQDKDKRGGIFDAVFTRGDQTTLLTARHDLKNKGLNDISTIIKQELTEGRALALSHTYANVSISHVINLWGADFNAEGNLEAIYVTDSDANASIGMKKYFVGINAHGHVAISAKKIEGENIGAQVLGLFTLSSGKDIWQKLS

SEQ ID NO: 13 - protein, 312 aa, Streptococcus pyogenes
DDYQRNATEAYAKEVPHQITSVWTKGVTPPEQFTQGEDVIHAPYLAHQGWYDITKAFDGKDNLLCGAATAGNMLHWWFDQNKTEIEAYLSKHPEKQKIIINNQELFDLKAAIDTKDSQTNSQLFNYFRDKAFPNLSARQLGVMPDLVLDMFINGYYLNVFKTQSTDVNRPYQDKDKRGGIFDAVFTRGDQTTLLTARHDLKNKGLNDISTIIKQELTEGRALALSHTYANVSISHVINLWGADFNAEGNLEAIYVTDSDANASIGMKKYFVGINAHGHVAISAKKIEGENIGAQVLGLFTLSSGKDIWQKLS

SEQ ID NO: 14 - protein, 312 aa, Streptococcus pyogenes
DDYQRNATEAYAKEVPHQITSVWTKGVTPPEQFTQGEDVIHAPYLAHQGWYDITKAFDGKDNLLCGAATAGNMLHWWFDQNKTEIEAYLSKHPEKQKIIFRNQELFDLKAAIDTKDSQTNSQLFNYFRDKAFPNLSARQLGVMPDLVLDMFINGYYLNVFKTQSTDVNRPYQDKDKRGGIFDAVFTRGDQTTLLTARHDLKNKGLNDISTIIKQELTEGRALALSHTYANVSISHVINLWGADFNAEGNLEAIYVTDSDANASIGMKKYFVGINAHGHVAISAKKIEGENIGAQVLGLFTLSSGKDIWQKLS

SEQ ID NO: 15 - protein, 312 aa, Streptococcus pyogenes
DDYQRNATEAYAKEVPHQITSVWTKGVTPPEQFTQGEDVIHAPYLAHQGWYDITKAFDGKDNLLCGAATAGNMLHWWFDQNKTEIEAYLSKHPEKQKIIIRNQELFDLKAAIDTKDSQTNSQLFNYFRDKAFPNLSARQLGVMPDLVLDMFINGYYLNVFKTQSTDVNRPYQDKDKRGGIFDAVFTRGDQTTLLTARHDLKNKGLNDISTIIKQELTEGRALALSHTYANVSISHVINLWGADFNAEGNLEAIYVTDSDANASIGMKKYFVGINAHGHVAISAKKIEGENIGAQVLGLFTLSSGKDIWQKLS

SEQ ID NO: 16 - protein, 312 aa, Streptococcus pyogenes
DDYQRNATEAYAKEVPHQITSVWTKGVTPPEQFTQGEDVIHAPYLANQGWYDITKAFDGKDNLLCGAATAGNMLHWWFDQNKTEIEAYLSKHPEKQKIIFRNQELFDLKEAIRTKDSQTNSQLFEYFRDKAFPYLSARQLGVMPDLVLDMFINGYYLNVFKTQSTDVKRPYQDKDKRGGIFDAVFTRGNQTTLLTARHDLKNKGLNDISTIIKEELTKGRALALSHTYANVSISHVINLWGADFNAEGNLEAIYVTDSDANASIGMKKYFVGINKHGHVAISAKKIEGENIGAQVLGLFTLSSGKDIWQKLN

SEQ ID NO: 17 - protein, 292 aa, Streptococcus pyogenes
SVWTKGVTPPEQFTQGEDVIHAPYLAHQGWYDITKAFDGKDNLLCGAATAGNMLHWWFDQNKTEIEAYLSKHPEKQKIIFRNQELFDLKAAIDTKDSQTNSQLFNYFRDKAFPNLSARQLGVMPDLVLDMFINGYYLNVFKTQSTDVNRPYQDKDKRGGIFDAVFTRGNQTTLLTARHDLKNKGLNDISTIIKQELTEGRALALSHTYANVSISHVINLWGADFNAEGNLEAIYVTDSDANASIGMKKYFVGINAHGHVAISAKKIEGENIGAQVLGLFTLSSGKDIWQKLS

SEQ ID NO: 18 - protein, 312 aa, Streptococcus pyogenes
DDYQRNATEAYAKEVPHQITSVWTKGVTPPEQFTQGEDVIHAPYLAHQGWYDITKAFDGADNLLCGAATAGNMLHWWFDQNKTEIEAYLSKHPEKQKIIFRNQELFDLKAAIDTKDSQTNSQLFNYFRDKAFPNLSARQLGVMPDLVLDMFINGYYLNVFKTQSTDVNRPYQDKDKRGGIFDAVFTRGNQTTLLTARHDLKNKGLNDISTIIKQELTEGRALALSHTYANVSISHVINLWGADFNAEGNLEAIYVTDSDANASIGMKKYFVGINAHGHVAISAKKIEGENIGAQVLGLFTLSSGKDIWQKLS

SEQ ID NO: 19 - protein, 292 aa, Streptococcus pyogenes
SVWTKGVTPPEQFTQGEDVIHAPYLAHQGWYDITKAFDGADNLLCGAATAGNMLHWWFDQNKTEIEAYLSKHPEKQKIIFRNQELFDLKAAIDTKDSQTNSQLFNYFRDKAFPNLSARQLGVMPDLVLDMFINGYYLNVFKTQSTDVNRPYQDKDKRGGIFDAVFTRGNQTTLLTARHDLKNKGLNDISTIIKQELTEGRALALSHTYANVSISHVINLWGADFNAEGNLEAIYVTDSDANASIGMKKYFVGINAHGHVAISAKKIEGENIGAQVLGLFTLSSGKDIWQKLS

SEQ ID NO: 20 - protein, 312 aa, Streptococcus pyogenes
DDYQRNATEAYAKEVPHQITSVWTKGVTPPEQFTQGEDVIHAPYLAHQGWYDITKAFDGKDNLLCGAATAGNMLHWWFDQNKTEIEAYLSKHPEKQKIIFRNQELFDLKAAIDTKDSQTNSQLFNYFRDKAFPNLSARQLGVMPDLVLDMFINGYYLNVFKTQSTDVNRPYQDKDKRGGIFDAVFTRGNQTTLLTARHDLKNKGLNDISTIIKQELTEGRALALSHTYANVSISHVINLWGADFNAEGNLEAIYVTDSDANASIGMKKYFVGINAHGHVAISAKKIEGENIGAQVLGLFTLSSGKDIWQKLS

SEQ ID NO: 21 - protein, 312 aa, Streptococcus pyogenes
DDYQRNATEAYAKEVPHQITSVWTKGVTPLTPEQFTQGEDVFHAPYVANQGWYDITKAFDGKDNLLCGAATAGNMLHWWFDQNKDQIKRYLEEHPEKQKINFNGENMFDVKKAIDTKNHQLDSKLFNYFKEKAFPYLSAKHLGVFPDHVIDMFINGYRLSLTNHGPTPVKEGSKDPRGGIFDAVFTRGNQSKLLTSRHDFKNKNLNDISTIIKQELTKGKALGLSHTYANVRINHVINLWGADFNAEGNLEAIYVTDSDSNASIGMKKYFVGVNAHGHVAISAKKIEGENIGAQVLGLFTLSTGQDSWQKLS

SEQ ID NO: 22 - protein, 312 aa, Streptococcus pyogenes
DDYQRNATEAYAKEVPHQITSVWTKGVTPLTPEQFTQGEDVFHAPYVANQGWYDITKAFDGKDNLLCGAATAGNMLHWWFDQNKDQIKRYLEEHPEKQKINFRGENMFDVKEAIRTKNHQLDSKLFEYFKEKAFPYLSAKHLGVFPDHVIDMFINGYRLSLTNHGPTPVKKGSKDPRGGIFDAVFTRGNQSKLLTSRHDFKNKNLNDISTIIKSELTNGKALGLSHTYANVRINHVINLWGADFNAEGNLEAIYVTDSDSNASIGMKKYFVGVNKHGHVAISAKKIEGENIGAQVLGLFTLSTGQDSWQKLN

SEQ ID NO: 23 - protein, 312 aa, Streptococcus pyogenes
DDYQRNATEAYAKEVPHQITSVWTKGVTPLTPEQFTQGEDVFHAPYVANQGWYDITKTFNGKDDLLCGAATAGNMLHWWFDQNKDQIKRYLEEHPEKQKINFNGEQMFDVKEAIDTKNHQLDSKLFEYFKEKAFPYLSTKHLGVFPDHVIDMFINGYRLSLTNHGPTPVKEGSKDPRGGIFDAVFTRGNQSKLLTSRHDFKEKNLKEISDLIKQELTEGKALGLSHTYANVRINHVINLWGADFDAEGNLKAIYVTDSDSNASIGMKKYFVGVNAAGKVAISAKKIEGENIGAQVLGLFTLSTGQDSWNQTS

SEQ ID NO: 24 - protein, 312 aa, Streptococcus pyogenes
DDYQRNATEAYAKEVPHQITSVWTKGVTPLTPEQFTQGEDVFHAPYVANQGWYDITKTFNGKDDLLCGAATAGNMLHWWFDQNKDQIKRYLEEHPEKQKINFRGEQMFDVKEAIRTKNHQLDSKLFEYFKEKAFPYLSTKHLGVFPDHVIDMFINGYRLSLTNHGPTPVKKGSKDPRGGIFDAVFTRGNQSKLLTSRHDFKEKNLKEISDLIKEELTKGKALGLSHTYANVRINHVINLWGADFDAEGNLKAIYVTDSDSNASIGMKKYFVGVNKAGKVAISAKKIEGENIGAQVLGLFTLSTGQDSWNQTN

SEQ ID NO: 25 - protein, 310 aa, Streptococcus pyogenes
DDYQRNATEAYAKEVPHQITSVWTKGVTPPEQFTQGEDVIHAPYVANQGWYDITKAFDGKDNLLCGAATAGNMLHWWFDQNKDQIKRYLEEHPEKQKINFRGEQMFDVKKAIDTKNHQLDSKLFNYFKEKAFPGLSARRIGVFPDHVIDMFINGYRLSLTNHGPTPVKEGSKDPRGGIFDAVFTRGNQSKLLTSRHDFKNKNLNDISTIIKQELTKGKALGLSHTYANVSINHVINLWGADFNAEGNLEAIYVTDSDSNASIGMKKYFVGVNAHGHVAISAKKIEGENIGAQVLGLFTLSTGQDSWQKLS

SEQ ID NO: 26 - protein, 320 aa, Streptococcus pyogenes
MDSFSANQEIRYSEVTPYHVTSVWTKGVTPPANFTQGEDVFHAPYVANQGWYDITKTFNGKDDLLCGAATAGNMLHWWFDQNKDQIKRYLEEHPEKQKINFNGEQMFDVKEAIDTKNHQLDSKLFEYFKEKAFPYLSTKHLGVFPDHVIDMFINGYRLSLTNHGPTPVKEGSKDPRGGIFDAVFTRGDQSKLLTSRHDFKEKNLKEISDLIKKELTEGKALGLSHTYANVRINHVINLWGADFDSNGNLKAIYVTDSDSNASIGMKKYFVGVNSAGKVAISAKEIKEDNIGAQVLGLFTLSTGQDSWNQTNGGGHHHHHH

SEQ ID NO: 27 - protein, 325 aa, Streptococcus pyogenes
MDDYQRNATEAYAKEVPHQITSVWTKGVTPLTPEQFRYNNEDVIHAPYLAHQGWYDITKAFDGKDNLLCGAATAGNMLHWWFDQNKTEIEAYLSKHPEKQKIIFNNQELFDLKAAIDTKDSQTNSQLFNYFRDKAFPNLSARQLGVMPDLVLDMFINGYYLNVFKTQSTDVNRPYQDKDKRGGIFDAVFTRGDQTTLLTARHDLKNKGLNDISTIIKQELTEGRALALSHTYANVSISHVINLWGADFNAEGNLEAIYVTDSDANASIGMKKYFVGINAHGHVAISAKKIEGENIGAQVLGLFTLSSGKDIWQKLSGGGHHHHHH

SEQ ID NO: 28 - protein, 323 aa, Streptococcus pyogenes
MDDYQRNATEAYAKEVPHQITSVWTKGVTPLTPEQFRYNNEDVFHAPYVANQGWYDITKAFDGKDNLLCGAATAGNMLHWWFDQNKDQIKRYLEEHPEKQKINFNGDNMFDVKKAIDTKNHQLDSKLFNYFKEKAFPGLSARRIGVFPDHVIDMFINGYRLSLTNHGPTPVKEGSKDPRGGIFDAVFTRGNQSKLLTSRHDFKNKNLNDISTIIKQELTKGKALGLSHTYANVSINHVINLWGADFNAEGNLEAIYVTDSDSNASIGMKKYFVGVNAHGHVAISAKKIEGENIGAQVLGLFTLSTGQDSWQKLSGGGHHHHHH

SEQ ID NO: 29 - protein, 11 aa, Streptococcus pyogenes
PLTPEQFRYNN

SEQ ID NO: 30 - protein, 8 aa, Streptococcus pyogenes
PPANFTQG

SEQ ID NO: 31 - protein, 20 aa, Streptococcus pyogenes
DDYQRNATEAYAKEVPHQIT

SEQ ID NO: 32 - protein, 20 aa, Streptococcus pyogenes
DSFSANQEIRYSEVTPYHVT

SEQ ID NO: 33 - DNA, 963 bp, Streptococcus pyogenes
atggatagtttttctgctaatcaagagattagatattcggaagtaacaccttatcacgttacttccgtttggaccaaaggagttactcctccagcaaacttcactcaaggtgaagatgtttttcacgctccttatgttgctaaccaaggatggtatgatattaccaaaacattcaatggaaaagacgatcttctttgcggggctgccacagcagggaatatgcttcactggtggttcgatcaaaacaaagaccaaattaaacgttatttggaagagcatccagaaaagcaaaaaataaacttcaatggcgaacagatgtttgacgtaaaagaagctatcgacactaaaaaccaccagctagatagtaaattatttgaatattttaaagaaaaagctttcccttatctatctactaaacacctaggagttttccctgatcatgtaattgatatgttcattaacggctaccgccttagtctaactaaccacggtccaacgccagtaaaagaaggtagtaaagatccccgaggtggtatttttgacgccgtatttacaagaggtgatcaaagtaagctattgacaagtcgtcatgattttaaagaaaaaaatctcaaagaaatcagtgatctcattaagaaagagttaaccgaaggcaaggctctaggcctatcacacacctacgctaacgtacgcatcaaccatgttataaacctgtggggagctgactttgattctaacgggaaccttaaagctatttatgtaacagactctgatagtaatgcatctattggtatgaagaaatactttgttggtgttaattccgctggaaaagtagctatttctgctaaagaaataaaagaagataatataggtgctcaagtactagggttatttacactttcaacagggcaagatagttggaatcagaccaatggcggtggccatcatcaccatcaccactaa

SEQ ID NO: 34 - DNA, 978 bp, Streptococcus pyogenes
atggacgattaccaaaggaatgctacggaagcttatgccaaagaagtaccacatcagatcacttctgtatggaccaaaggtgttacaccactaacacccgagcagtttcgatataataacgaagatgtgatccatgcgccatatcttgctcatcaaggctggtacgatatcaccaaggccttcgatgggaaggataatctcttgtgtggcgcagcaacggcaggtaatatgctgcattggtggtttgatcaaaataaaacagagattgaagcctatttaagtaaacaccctgaaaagcaaaaaatcatttttaacaaccaagagctatttgatttgaaagctgctatcgataccaaggacagtcaaaccaatagtcagctttttaattattttagagataaagcctttccaaatctatcagcacgtcaactcggggttatgcctgatcttgttctagatatgtttatcaatggttactacttaaatgtgtttaaaacacagtctactgatgtcaatcgaccttatcaggacaaggacaaacgaggtggtattttcgatgctgttttcaccagaggagatcagacaacgctcttgacagctcgtcatgatttaaaaaataaaggactaaatgacatcagcaccattatcaagcaagaactgactgaaggaagagcccttgctttatcacatacctacgccaatgttagcattagccatgtgattaacttgtggggagctgattttaatgctgaaggaaaccttgaggccatctatgtcacagactcagatgctaatgcgtctattggtatgaaaaaatattttgtcggcattaatgctcatggacatgtcgccatttctgccaagaaaatagaaggagaaaacattggcgctcaagtattaggcttatttacgctttccagtggcaaggacatttggcagaaactgagcggcggtggccatcatcaccatcaccactaa

SEQ ID NO: 35 - DNA, 972 bp, Streptococcus pyogenes
atggatgattatcagcgcaacgcgaccgaagcgtatgcgaaagaagtgccgcatcagattaccagcgtgtggaccaaaggcgtgaccccgctgaccccggaacagtttcgctataacaacgaagatgtgtttcatgcgccgtatgtggcgaaccagggctggtatgatattaccaaagcgtttgatggcaaagataacctgctgtgcggcgcggcgaccgcgggcaacatgctgcattggtggtttgatcagaacaaagatcagattaaacgctatctggaagaacatccggaaaaacagaaaattaactttaacggcgataacatgtttgatgtgaaaaaagcgattgataccaaaaaccatcagctggatagcaaactgtttaactattttaaagaaaaagcgtttccgggcctgagcgcgcgccgcattggcgtgtttccggatcatgtgattgatatgtttattaacggctatcgcctgagcctgaccaaccatggcccgaccccggtgaaagaaggcagcaaagatccgcgcggcggcatttttgatgcggtgtttacccgcggcaaccagagcaaactgctgaccagccgccatgattttaaaaacaaaaacctgaacgatattagcaccattattaaacaggaactgaccaaaggcaaagcgctgggcctgagccatacctatgcgaacgtgagcattaaccatgtgattaacctgtggggcgcggattttaacgcggaaggcaacctggaagcgatttatgtgaccgatagcgatagcaacgcgagcattggcatgaaaaaatattttgtgggcgtgaacgcgcatggccatgtggcgattagcgcgaaaaaaattgaaggcgaaaacattggcgcgcaggtgctgggcctgtttaccctgagcaccggccaggatagctggcagaaactgagcggcggtggccatcatcaccatcaccactaa

SEQ ID NO: 36 - DNA, 978 bp, Streptococcus pyogenes
atggatgattatcagcgcaacgcgaccgaagcgtatgcgaaagaagtgccgcatcagattaccagcgtgtggaccaaaggcgtgaccccgctgaccccggaacagtttcgctataacaacgaagatgtgattcatgcgccgtatctggcgaaccagggctggtatgatattaccaaagcgtttgatggcaaagataacctgctgtgcggcgcggcgaccgcgggcaacatgctgcattggtggtttgatcagaacaaaaccgaaattgaagcgtatctgagcaaacatccggaaaaacagaaaattatttttcgcaaccaggaactgtttgatctgaaagaagcgattcgcaccaaagatagccagaccaacagccagctgtttgaatattttcgcgataaagcgtttccgtatctgagcgcgcgccagctgggcgtgatgccggatctggtgctggatatgtttattaacggctattatctgaacgtgtttaaaacccagagcaccgatgtgaaacgcccgtatcaggataaagataaacgcggcggcatttttgatgcggtgtttacccgcggcaaccagaccaccctgctgaccgcgcgccatgatctgaaaaacaaaggcctgaacgatattagcaccattattaaagaagaactgaccaaaggccgcgcgctggcgctgagccatacctatgcgaacgtgagcattagccatgtgattaacctgtggggcgcggattttaacgcggaaggcaacctggaagcgatttatgtgaccgatagcgatgcgaacgcgagcattggcatgaaaaaatattttgtgggcattaacaaacatggccatgtggcgattagcgcgaaaaaaattgaaggcgaaaacattggcgcgcaggtgctgggcctgtttaccctgagcagcggcaaagatatttggcagaaactgaacggcggtggccatcatcaccatcaccactaa

SEQ ID NO: 37 - DNA, 978 bp, Streptococcus pyogenes
atggatgattatcagcgcaacgcgaccgaagcgtatgcgaaagaagtgccgcatcagattaccagcgtgtggaccaaaggcgtgaccccgctgaccccggaacagtttcgctataacaacgaagatgtgattcatgcgccgtatctggcgcatcagggctggtatgatattaccaaaacctttaacggcaaagataacctgctgtgcggcgcggcgaccgcgggcaacatgctgcattggtggtttgatcagaacaaaaccgaaattgaagcgtatctgagcaaacatccggaaaaacagaaaattatttttaacaacgaagaactgtttgatctgaaagcggcgattgataccaaagatagccagaccaacagccagctgtttaactattttaaagaaaaagcgtttccgaacctgagcacccgccagctgggcgtgatgccggatctggtgctggatatgtttattaacggctattatctgaacgtgtttaaaacccagagcaccgatgtgaaccgcccgtatcaggataaagataaacgcggcggcatttttgatgcggtgtttacccgcggcaaccagaccaccctgctgaccgcgcgccatgattttaaagaaaaaggcctgaaagatattagcaccattattaaacaggaactgaccgaaggccgcgcgctggcgctgagccatacctatgcgaacgtgagcattagccatgtgattaacctgtggggcgcggattttgatgcggaaggcaacctgaaagcgatttatgtgaccgatagcgatgcgaacgcgagcattggcatgaaaaaatattttgtgggcattaacgcgcatggcaaagtggcgattagcgcgaaaaaaattgaaggcgaaaacattggcgcgcaggtgctgggcctgtttaccctgagcagcggcaaagatatttggcagcagctgagcggcggtggccatcatcaccatcaccactaa

SEQ ID NO: 38 - DNA, 978 bp, Streptococcus pyogenes
atggatagctttagcgcgaaccaggaaattcgctatagcgaagtgaccccgtatcatgtgaccagcgtgtggaccaaaggcgtgaccccgctgaccccggaacagtttcgctataacaacgaagatgtgattcatgcgccgtatctggcgcatcagggctggtatgatattaccaaagcgtttgatggcaaagataacctgctgtgcggcgcggcgaccgcgggcaacatgctgcattggtggtttgatcagaacaaaaccgaaattgaagcgtatctgagcaaacatccggaaaaacagaaaattatttttaacaaccaggaactgtttgatctgaaagcggcgattgataccaaagatagccagaccaacagccagctgtttaactattttcgcgataaagcgtttccgaacctgagcgcgcgccagctgggcgtgatgccggatctggtgctggatatgtttattaacggctattatctgaacgtgtttaaaacccagagcaccgatgtgaaccgcccgtatcaggataaagataaacgcggcggcatttttgatgcggtgtttacccgcggcgatcagaccaccctgctgaccgcgcgccatgatctgaaaaacaaaggcctgaacgatattagcaccattattaaacaggaactgaccgaaggccgcgcgctggcgctgagccatacctatgcgaacgtgagcattagccatgtgattaacctgtggggcgcggattttaacgcggaaggcaacctggaagcgatttatgtgaccgatagcgatgcgaacgcgagcattggcatgaaaaaatattttgtgggcattaacgcgcatggccatgtggcgattagcgcgaaaaaaattgaaggcgaaaacattggcgcgcaggtgctgggcctgtttaccctgagcagcggcaaagatatttggcagaaactgagcggcggtggccatcatcaccatcaccactaa

SEQ ID NO: 39 - DNA, 918 bp, Streptococcus pyogenes
atgagcgtgtggaccaaaggcgtgaccccgctgaccccggaacagtttcgctataacaacgaagatgtgattcatgcgccgtatctggcgcatcagggctggtatgatattaccaaagcgtttgatggcaaagataacctgctgtgcggcgcggcgaccgcgggcaacatgctgcattggtggtttgatcagaacaaaaccgaaattgaagcgtatctgagcaaacatccggaaaaacagaaaattatttttaacaaccaggaactgtttgatctgaaagcggcgattgataccaaagatagccagaccaacagccagctgtttaactattttcgcgataaagcgtttccgaacctgagcgcgcgccagctgggcgtgatgccggatctggtgctggatatgtttattaacggctattatctgaacgtgtttaaaacccagagcaccgatgtgaaccgcccgtatcaggataaagataaacgcggcggcatttttgatgcggtgtttacccgcggcgatcagaccaccctgctgaccgcgcgccatgatctgaaaaacaaaggcctgaacgatattagcaccattattaaacaggaactgaccgaaggccgcgcgctggcgctgagccatacctatgcgaacgtgagcattagccatgtgattaacctgtggggcgcggattttaacgcggaaggcaacctggaagcgatttatgtgaccgatagcgatgcgaacgcgagcattggcatgaaaaaatattttgtgggcattaacgcgcatggccatgtggcgattagcgcgaaaaaaattgaaggcgaaaacattggcgcgcaggtgctgggcctgtttaccctgagcagcggcaaagatatttggcagaaactgagcggcggtggccatcatcaccatcaccactaa

SEQ ID NO: 40 - DNA, 975 bp, Streptococcus pyogenes
atggacgattaccaaaggaatgctacggaagcttatgccaaagaagtaccacatcagatcacttctgtatggaccaaaggtgttacaccactaacacccgagcagtttactcaaggtgaagatgtgatccatgcgccatatcttgctcatcaaggctggtacgatatcaccaaggccttcgatgggaaggataatctcttgtgtggcgcagcaacggcaggtaatatgctgcattggtggtttgatcaaaataaaacagagattgaagcctatttaagtaaacaccctgaaaagcaaaaaatcatttttaacaaccaagagctatttgatttgaaagctgctatcgataccaaggacagtcaaaccaatagtcagctttttaattattttagagataaagcctttccaaatctatcagcacgtcaactcggggttatgcctgatcttgttctagatatgtttatcaatggttactacttaaatgtgtttaaaacacagtctactgatgtcaatcgaccttatcaggacaaggacaaacgaggtggtattttcgatgctgttttcaccagaggagatcagacaacgctcttgacagctcgtcatgatttaaaaaataaaggactaaatgacatcagcaccattatcaagcaagaactgactgaaggaagagcccttgctttatcacatacctacgccaatgttagcattagccatgtgattaacttgtggggagctgattttaatgctgaaggaaaccttgaggccatctatgtcacagactcagatgctaatgcgtctattggtatgaaaaaatattttgtcggcattaatgctcatggacatgtcgccatttctgccaagaaaatagaaggagaaaacattggcgctcaagtattaggcttatttacgctttccagtggcaaggacatttggcagaaactgagcggcggtggccatcatcaccatcaccactaa

SEQ ID NO: 41 - DNA, 969 bp, Streptococcus pyogenes
atggacgattaccaaaggaatgctacggaagcttatgccaaagaagtaccacatcagatcacttctgtatggaccaaaggtgttacaccacccgagcagtttactcaaggtgaagatgtgatccatgcgccatatcttgctcatcaaggctggtacgatatcaccaaggccttcgatgggaaggataatctcttgtgtggcgcagcaacggcaggtaatatgctgcattggtggtttgatcaaaataaaacagagattgaagcctatttaagtaaacaccctgaaaagcaaaaaatcatttttaacaaccaagagctatttgatttgaaagctgctatcgataccaaggacagtcaaaccaatagtcagctttttaattattttagagataaagcctttccaaatctatcagcacgtcaactcggggttatgcctgatcttgttctagatatgtttatcaatggttactacttaaatgtgtttaaaacacagtctactgatgtcaatcgaccttatcaggacaaggacaaacgaggtggtattttcgatgctgttttcaccagaggagatcagacaacgctcttgacagctcgtcatgatttaaaaaataaaggactaaatgacatcagcaccattatcaagcaagaactgactgaaggaagagcccttgctttatcacatacctacgccaatgttagcattagccatgtgattaacttgtggggagctgattttaatgctgaaggaaaccttgaggccatctatgtcacagactcagatgctaatgcgtctattggtatgaaaaaatattttgtcggcattaatgctcatggacatgtcgccatttctgccaagaaaatagaaggagaaaacattggcgctcaagtattaggcttatttacgctttccagtggcaaggacatttggcagaaactgagcggcggtggccatcatcaccatcaccactaa

SEQ ID NO: 42 - DNA, 972 bp, Streptococcus pyogenes
atggacgattaccaaaggaatgctacggaagcttatgccaaagaagtaccacatcagatcacttctgtatggaccaaaggtgttacaccacccgagcagtttcgatataataacgaagatgtgatccatgcgccatatcttgctcatcaaggctggtacgatatcaccaaggccttcgatgggaaggataatctcttgtgtggcgcagcaacggcaggtaatatgctgcattggtggtttgatcaaaataaaacagagattgaagcctatttaagtaaacaccctgaaaagcaaaaaatcatttttaacaaccaagagctatttgatttgaaagctgctatcgataccaaggacagtcaaaccaatagtcagctttttaattattttagagataaagcctttccaaatctatcagcacgtcaactcggggttatgcctgatcttgttctagatatgtttatcaatggttactacttaaatgtgtttaaaacacagtctactgatgtcaatcgaccttatcaggacaaggacaaacgaggtggtattttcgatgctgttttcaccagaggagatcagacaacgctcttgacagctcgtcatgatttaaaaaataaaggactaaatgacatcagcaccattatcaagcaagaactgactgaaggaagagcccttgctttatcacatacctacgccaatgttagcattagccatgtgattaacttgtggggagctgattttaatgctgaaggaaaccttgaggccatctatgtcacagactcagatgctaatgcgtctattggtatgaaaaaatattttgtcggcattaatgctcatggacatgtcgccatttctgccaagaaaatagaaggagaaaacattggcgctcaagtattaggcttatttacgctttccagtggcaaggacatttggcagaaactgagcggcggtggccatcatcaccatcaccactaa

SEQ ID NO: 43 - DNA, 969 bp, Streptococcus pyogenes
atggacgattaccaaaggaatgctacggaagcttatgccaaagaagtaccacatcagatcacttctgtatggaccaaaggtgttacaccacccgagcagtttactcaaggtgaagatgtgatccatgcgccatatcttgctcatcaaggctggtacgatatcaccaaggccttcgatgggaaggataatctcttgtgtggcgcagcaacggcaggtaatatgctgcattggtggtttgatcaaaataaaacagagattgaagcctatttaagtaaacaccctgaaaagcaaaaaatcattattaacaaccaagagctatttgatttgaaagctgctatcgataccaaggacagtcaaaccaatagtcagctttttaattattttagagataaagcctttccaaatctatcagcacgtcaactcggggttatgcctgatcttgttctagatatgtttatcaatggttactacttaaatgtgtttaaaacacagtctactgatgtcaatcgaccttatcaggacaaggacaaacgaggtggtattttcgatgctgttttcaccagaggagatcagacaacgctcttgacagctcgtcatgatttaaaaaataaaggactaaatgacatcagcaccattatcaagcaagaactgactgaaggaagagcccttgctttatcacatacctacgccaatgttagcattagccatgtgattaacttgtggggagctgattttaatgctgaaggaaaccttgaggccatctatgtcacagactcagatgctaatgcgtctattggtatgaaaaaatattttgtcggcattaatgctcatggacatgtcgccatttctgccaagaaaatagaaggagaaaacattggcgctcaagtattaggcttatttacgctttccagtggcaaggacatttggcagaaactgagcggcggtggccatcatcaccatcaccactaa

SEQ ID NO: 44 - DNA, 969 bp, Streptococcus pyogenes
atggacgattaccaaaggaatgctacggaagcttatgccaaagaagtaccacatcagatcacttctgtatggaccaaaggtgttacaccacccgagcagtttactcaaggtgaagatgtgatccatgcgccatatcttgctcatcaaggctggtacgatatcaccaaggccttcgatgggaaggataatctcttgtgtggcgcagcaacggcaggtaatatgctgcattggtggtttgatcaaaataaaacagagattgaagcctatttaagtaaacaccctgaaaagcaaaaaatcatttttcgtaaccaagagctatttgatttgaaagctgctatcgataccaaggacagtcaaaccaatagtcagctttttaattattttagagataaagcctttccaaatctatcagcacgtcaactcggggttatgcctgatcttgttctagatatgtttatcaatggttactacttaaatgtgtttaaaacacagtctactgatgtcaatcgaccttatcaggacaaggacaaacgaggtggtattttcgatgctgttttcaccagaggagatcagacaacgctcttgacagctcgtcatgatttaaaaaataaaggactaaatgacatcagcaccattatcaagcaagaactgactgaaggaagagcccttgctttatcacatacctacgccaatgttagcattagccatgtgattaacttgtggggagctgattttaatgctgaaggaaaccttgaggccatctatgtcacagactcagatgctaatgcgtctattggtatgaaaaaatattttgtcggcattaatgctcatggacatgtcgccatttctgccaagaaaatagaaggagaaaacattggcgctcaagtattaggcttatttacgctttccagtggcaaggacatttggcagaaactgagcggcggtggccatcatcaccatcaccactaa

SEQ ID NO: 45 - DNA, 969 bp, Streptococcus pyogenes
atggacgattaccaaaggaatgctacggaagcttatgccaaagaagtaccacatcagatcacttctgtatggaccaaaggtgttacaccacccgagcagtttactcaaggtgaagatgtgatccatgcgccatatcttgctcatcaaggctggtacgatatcaccaaggccttcgatgggaaggataatctcttgtgtggcgcagcaacggcaggtaatatgctgcattggtggtttgatcaaaataaaacagagattgaagcctatttaagtaaacaccctgaaaagcaaaaaatcattattcgtaaccaagagctatttgatttgaaagctgctatcgataccaaggacagtcaaaccaatagtcagctttttaattattttagagataaagcctttccaaatctatcagcacgtcaactcggggttatgcctgatcttgttctagatatgtttatcaatggttactacttaaatgtgtttaaaacacagtctactgatgtcaatcgaccttatcaggacaaggacaaacgaggtggtattttcgatgctgttttcaccagaggagatcagacaacgctcttgacagctcgtcatgatttaaaaaataaaggactaaatgacatcagcaccattatcaagcaagaactgactgaaggaagagcccttgctttatcacatacctacgccaatgttagcattagccatgtgattaacttgtggggagctgattttaatgctgaaggaaaccttgaggccatctatgtcacagactcagatgctaatgcgtctattggtatgaaaaaatattttgtcggcattaatgctcatggacatgtcgccatttctgccaagaaaatagaaggagaaaacattggcgctcaagtattaggcttatttacgctttccagtggcaaggacatttggcagaaactgagcggcggtggccatcatcaccatcaccactaa

SEQ ID NO: 46 - DNA, 969 bp, Streptococcus pyogenes
atggatgattatcagcgcaacgcgaccgaagcgtatgcgaaagaagtgccgcatcagattaccagcgtgtggaccaaaggcgtgaccccgccggaacagtttactcaaggtgaagatgtgattcatgcgccgtatctggcgaaccagggctggtatgatattaccaaagcgtttgatggcaaagataacctgctgtgcggcgcggcgaccgcgggcaacatgctgcattggtggtttgatcagaacaaaaccgaaattgaagcgtatctgagcaaacatccggaaaaacagaaaattatttttcgcaaccaggaactgtttgatctgaaagaagcgattcgcaccaaagatagccagaccaacagccagctgtttgaatattttcgcgataaagcgtttccgtatctgagcgcgcgccagctgggcgtgatgccggatctggtgctggatatgtttattaacggctattatctgaacgtgtttaaaacccagagcaccgatgtgaaacgcccgtatcaggataaagataaacgcggcggcatttttgatgcggtgtttacccgcggcaaccagaccaccctgctgaccgcgcgccatgatctgaaaaacaaaggcctgaacgatattagcaccattattaaagaagaactgaccaaaggccgcgcgctggcgctgagccatacctatgcgaacgtgagcattagccatgtgattaacctgtggggcgcggattttaacgcggaaggcaacctggaagcgatttatgtgaccgatagcgatgcgaacgcgagcattggcatgaaaaaatattttgtgggcattaacaaacatggccatgtggcgattagcgcgaaaaaaattgaaggcgaaaacattggcgcgcaggtgctgggcctgtttaccctgagcagcggcaaagatatttggcagaaactgaacggcggtggccatcatcaccatcaccactaa

SEQ ID NO: 47 - DNA, 909 bp, Streptococcus pyogenes
atgtctgtatggaccaaaggtgttacaccacccgagcagtttactcaaggtgaagatgtgatccatgcgccatatcttgctcatcaaggctggtacgatatcaccaaggccttcgatgggaaggataatctcttgtgtggcgcagcaacggcaggtaatatgctgcattggtggtttgatcaaaataaaacagagattgaagcctatttaagtaaacaccctgaaaagcaaaaaatcatttttcgtaaccaagagctatttgatttgaaagctgctatcgataccaaggacagtcaaaccaatagtcagctttttaattattttagagataaagcctttccaaatctatcagcacgtcaactcggggttatgcctgatcttgttctagatatgtttatcaatggttactacttaaatgtgtttaaaacacagtctactgatgtcaatcgaccttatcaggacaaggacaaacgaggtggtattttcgatgctgttttcaccagaggaaaccagacaacgctcttgacagctcgtcatgatttaaaaaataaaggactaaatgacatcagcaccattatcaagcaagaactgactgaaggaagagcccttgctttatcacatacctacgccaatgttagcattagccatgtgattaacttgtggggagctgattttaatgctgaaggaaaccttgaggccatctatgtcacagactcagatgctaatgcgtctattggtatgaaaaaatattttgtcggcattaatgctcatggacatgtcgccatttctgccaagaaaatagaaggagaaaacattggcgctcaagtattaggcttatttacgctttccagtggcaaggacatttggcagaaactgagcggcggtggccatcatcaccatcaccactaa

SEQ ID NO: 48 - DNA, 969 bp, Streptococcus pyogenes
atggacgattaccaaaggaatgctacggaagcttatgccaaagaagtaccacatcagatcacttctgtatggaccaaaggtgttacaccacccgagcagtttactcaaggtgaagatgtgatccatgcgccatatcttgctcatcaaggctggtacgatatcaccaaggccttcgatggggcggataatctcttgtgtggcgcagcaacggcaggtaatatgctgcattggtggtttgatcaaaataaaacagagattgaagcctatttaagtaaacaccctgaaaagcaaaaaatcatttttcgtaaccaagagctatttgatttgaaagctgctatcgataccaaggacagtcaaaccaatagtcagctttttaattattttagagataaagcctttccaaatctatcagcacgtcaactcggggttatgcctgatcttgttctagatatgtttatcaatggttactacttaaatgtgtttaaaacacagtctactgatgtcaatcgaccttatcaggacaaggacaaacgaggtggtattttcgatgctgttttcaccagaggaaatcagacaacgctcttgacagctcgtcatgatttaaaaaataaaggactaaatgacatcagcaccattatcaagcaagaactgactgaaggaagagcccttgctttatcacatacctacgccaatgttagcattagccatgtgattaacttgtggggagctgattttaatgctgaaggaaaccttgaggccatctatgtcacagactcagatgctaatgcgtctattggtatgaaaaaatattttgtcggcattaatgctcatggacatgtcgccatttctgccaagaaaatagaaggagaaaacattggcgctcaagtattaggcttatttacgctttccagtggcaaggacatttggcagaaactgagcggcggtggccatcatcaccatcaccactaa

SEQ ID NO: 49 - DNA, 909 bp, Streptococcus pyogenes
atgtctgtatggaccaaaggtgttacaccacccgagcagtttactcaaggtgaagatgtgatccatgcgccatatcttgctcatcaaggctggtacgatatcaccaaggccttcgatggggcggataatctcttgtgtggcgcagcaacggcaggtaatatgctgcattggtggtttgatcaaaataaaacagagattgaagcctatttaagtaaacaccctgaaaagcaaaaaatcatttttcgtaaccaagagctatttgatttgaaagctgctatcgataccaaggacagtcaaaccaatagtcagctttttaattattttagagataaagcctttccaaatctatcagcacgtcaactcggggttatgcctgatcttgttctagatatgtttatcaatggttactacttaaatgtgtttaaaacacagtctactgatgtcaatcgaccttatcaggacaaggacaaacgaggtggtattttcgatgctgttttcaccagaggaaatcagacaacgctcttgacagctcgtcatgatttaaaaaataaaggactaaatgacatcagcaccattatcaagcaagaactgactgaaggaagagcccttgctttatcacatacctacgccaatgttagcattagccatgtgattaacttgtggggagctgattttaatgctgaaggaaaccttgaggccatctatgtcacagactcagatgctaatgcgtctattggtatgaaaaaatattttgtcggcattaatgctcatggacatgtcgccatttctgccaagaaaatagaaggagaaaacattggcgctcaagtattaggcttatttacgctttccagtggcaaggacatttggcagaaactgagcggcggtggccatcatcaccatcaccactaa

SEQ ID NO: 50 - DNA, 969 bp, Streptococcus pyogenes
atggacgattaccaaaggaatgctacggaagcttatgccaaagaagtaccacatcagatcacttctgtatggaccaaaggtgttacaccacccgagcagtttactcaaggtgaagatgtgatccatgcgccatatcttgctcatcaaggctggtacgatatcaccaaggccttcgatgggaaggataatctcttgtgtggcgcagcaacggcaggtaatatgctgcattggtggtttgatcaaaataaaacagagattgaagcctatttaagtaaacaccctgaaaagcaaaaaatcatttttcgtaaccaagagctatttgatttgaaagctgctatcgataccaaggacagtcaaaccaatagtcagctttttaattattttagagataaagcctttccaaatctatcagcacgtcaactcggggttatgcctgatcttgttctagatatgtttatcaatggttactacttaaatgtgtttaaaacacagtctactgatgtcaatcgaccttatcaggacaaggacaaacgaggtggtattttcgatgctgttttcaccagaggaaaccagacaacgctcttgacagctcgtcatgatttaaaaaataaaggactaaatgacatcagcaccattatcaagcaagaactgactgaaggaagagcccttgctttatcacatacctacgccaatgttagcattagccatgtgattaacttgtggggagctgattttaatgctgaaggaaaccttgaggccatctatgtcacagactcagatgctaatgcgtctattggtatgaaaaaatattttgtcggcattaatgctcatggacatgtcgccatttctgccaagaaaatagaaggagaaaacattggcgctcaagtattaggcttatttacgctttccagtggcaaggacatttggcagaaactgagcggcggtggccatcatcaccatcaccactaa

SEQ ID NO: 51 - DNA, 969 bp, Streptococcus pyogenes
atggatgattatcagcgcaacgcgaccgaagcgtatgcgaaagaagtgccgcatcagattaccagcgtgtggaccaaaggcgtgaccccgctgaccccggaacagtttacccagggcgaagatgtgtttcatgcgccgtatgtggcgaaccagggctggtatgatattaccaaagcgtttgatggcaaagataacctgctgtgcggcgcggcgaccgcgggcaacatgctgcattggtggtttgatcagaacaaagatcagattaaacgctatctggaagaacatccggaaaaacagaaaattaactttaacggcgaaaacatgtttgatgtgaaaaaagcgattgataccaaaaaccatcagctggatagcaaactgtttaactattttaaagaaaaagcgtttccgtatctgagcgcgaaacatctgggcgtgtttccggatcatgtgattgatatgtttattaacggctatcgcctgagcctgaccaaccatggcccgaccccggtgaaagaaggcagcaaagatccgcgcggcggcatttttgatgcggtgtttacccgcggcaaccagagcaaactgctgaccagccgccatgattttaaaaacaaaaacctgaacgatattagcaccattattaaacaggaactgaccaaaggcaaagcgctgggcctgagccatacctatgcgaacgtgcgcattaaccatgtgattaacctgtggggcgcggattttaacgcggaaggcaacctggaagcgatttatgtgaccgatagcgatagcaacgcgagcattggcatgaaaaaatattttgtgggcgtgaacgcgcatggccatgtggcgattagcgcgaaaaaaattgaaggcgaaaacattggcgcgcaggtgctgggcctgtttaccctgagcaccggccaggatagctggcagaaactgagcggcggtggccatcatcaccatcaccactaa

SEQ ID NO: 52 - DNA, 969 bp, Streptococcus pyogenes
atggatgattatcagcgcaacgcgaccgaagcgtatgcgaaagaagtgccgcatcagattaccagcgtgtggaccaaaggcgtgaccccgctgaccccggaacagtttacccagggcgaagatgtgtttcatgcgccgtatgtggcgaaccagggctggtatgatattaccaaagcgtttgatggcaaagataacctgctgtgcggcgcggcgaccgcgggcaacatgctgcattggtggtttgatcagaacaaagatcagattaaacgctatctggaagaacatccggaaaaacagaaaattaactttcgcggcgaaaacatgtttgatgtgaaagaagcgattcgcaccaaaaaccatcagctggatagcaaactgtttgaatattttaaagaaaaagcgtttccgtatctgagcgcgaaacatctgggcgtgtttccggatcatgtgattgatatgtttattaacggctatcgcctgagcctgaccaaccatggcccgaccccggtgaaaaaaggcagcaaagatccgcgcggcggcatttttgatgcggtgtttacccgcggcaaccagagcaaactgctgaccagccgccatgattttaaaaacaaaaacctgaacgatattagcaccattattaaaagcgaactgaccaacggcaaagcgctgggcctgagccatacctatgcgaacgtgcgcattaaccatgtgattaacctgtggggcgcggattttaacgcggaaggcaacctggaagcgatttatgtgaccgatagcgatagcaacgcgagcattggcatgaaaaaatattttgtgggcgtgaacaaacatggccatgtggcgattagcgcgaaaaaaattgaaggcgaaaacattggcgcgcaggtgctgggcctgtttaccctgagcaccggccaggatagctggcagaaactgaacggcggtggccatcatcaccatcaccactaa

SEQ ID NO: 53 - DNA, 969 bp, Streptococcus pyogenes
atggatgattatcagcgcaacgcgaccgaagcgtatgcgaaagaagtgccgcatcagattaccagcgtgtggaccaaaggcgtgaccccgctgaccccggaacagtttacccagggcgaagatgtgtttcatgcgccgtatgtggcgaaccagggctggtatgatattaccaaaacctttaacggcaaagatgatctgctgtgcggcgcggcgaccgcgggcaacatgctgcattggtggtttgatcagaacaaagatcagattaaacgctatctggaagaacatccggaaaaacagaaaattaactttaacggcgaacagatgtttgatgtgaaagaagcgattgataccaaaaaccatcagctggatagcaaactgtttgaatattttaaagaaaaagcgtttccgtatctgagcaccaaacatctgggcgtgtttccggatcatgtgattgatatgtttattaacggctatcgcctgagcctgaccaaccatggcccgaccccggtgaaagaaggcagcaaagatccgcgcggcggcatttttgatgcggtgtttacccgcggcaaccagagcaaactgctgaccagccgccatgattttaaagaaaaaaacctgaaagaaattagcgatctgattaaacaggaactgaccgaaggcaaagcgctgggcctgagccatacctatgcgaacgtgcgcattaaccatgtgattaacctgtggggcgcggattttgatgcggaaggcaacctgaaagcgatttatgtgaccgatagcgatagcaacgcgagcattggcatgaaaaaatattttgtgggcgtgaacgcggcgggcaaagtggcgattagcgcgaaaaaaattgaaggcgaaaacattggcgcgcaggtgctgggcctgtttaccctgagcaccggccaggatagctggaaccagaccagcggcggtggccatcatcaccatcaccactaa

SEQ ID NO: 54 - DNA, 969 bp, Streptococcus pyogenes
atggatgattatcagcgcaacgcgaccgaagcgtatgcgaaagaagtgccgcatcagattaccagcgtgtggaccaaaggcgtgaccccgctgaccccggaacagtttacccagggcgaagatgtgtttcatgcgccgtatgtggcgaaccagggctggtatgatattaccaaaacctttaacggcaaagatgatctgctgtgcggcgcggcgaccgcgggcaacatgctgcattggtggtttgatcagaacaaagatcagattaaacgctatctggaagaacatccggaaaaacagaaaattaactttcgcggcgaacagatgtttgatgtgaaagaagcgattcgcaccaaaaaccatcagctggatagcaaactgtttgaatattttaaagaaaaagcgtttccgtatctgagcaccaaacatctgggcgtgtttccggatcatgtgattgatatgtttattaacggctatcgcctgagcctgaccaaccatggcccgaccccggtgaaaaaaggcagcaaagatccgcgcggcggcatttttgatgcggtgtttacccgcggcaaccagagcaaactgctgaccagccgccatgattttaaagaaaaaaacctgaaagaaattagcgatctgattaaagaagaactgaccaaaggcaaagcgctgggcctgagccatacctatgcgaacgtgcgcattaaccatgtgattaacctgtggggcgcggattttgatgcggaaggcaacctgaaagcgatttatgtgaccgatagcgatagcaacgcgagcattggcatgaaaaaatattttgtgggcgtgaacaaagcgggcaaagtggcgattagcgcgaaaaaaattgaaggcgaaaacattggcgcgcaggtgctgggcctgtttaccctgagcaccggccaggatagctggaaccagaccaacggcggtggccatcatcaccatcaccactaa

SEQ ID NO: 55 - DNA, 963 bp, Streptococcus pyogenes
atggatgattatcagcgcaacgcgaccgaagcgtatgcgaaagaagtgccgcatcagattaccagcgtgtggaccaaaggcgtgaccccgccggaacagtttactcaaggtgaagatgtgattcatgcgccgtatgtggcgaaccagggctggtatgatattaccaaagcgtttgatggcaaagataacctgctgtgcggcgcggcgaccgcgggcaacatgctgcattggtggtttgatcagaacaaagatcagattaaacgctatctggaagaacatccggaaaaacagaaaattaactttcgcggcgaacagatgtttgatgtgaaaaaagcgattgataccaaaaaccatcagctggatagcaaactgtttaactattttaaagaaaaagcgtttccgggcctgagcgcgcgccgcattggcgtgtttccggatcatgtgattgatatgtttattaacggctatcgcctgagcctgaccaaccatggcccgaccccggtgaaagaaggcagcaaagatccgcgcggcggcatttttgatgcggtgtttacccgcggcaaccagagcaaactgctgaccagccgccatgattttaaaaacaaaaacctgaacgatattagcaccattattaaacaggaactgaccaaaggcaaagcgctgggcctgagccatacctatgcgaacgtgagcattaaccatgtgattaacctgtggggcgcggattttaacgcggaaggcaacctggaagcgatttatgtgaccgatagcgatagcaacgcgagcattggcatgaaaaaatattttgtgggcgtgaacgcgcatggccatgtggcgattagcgcgaaaaaaattgaaggcgaaaacattggcgcgcaggtgctgggcctgtttaccctgagcaccggccaggatagctggcagaaactgagcggcggtggccatcatcaccatcaccactaa

SEQ ID NO: 56 - protein, 310 aa, Streptococcus pyogenes
DSFSANQEIRYSEVTPYHVTSVWTKGVTPPANFTQGEDVFHAPYVANQGWYDITKTFNGKDDLLCGAATAGNMLHWWFDQNKDQIKRYLEEHPEKQKINFRGEQMFDVKEAIDTKNHQLDSKLFEYFKEKAFPYLSTKHLGVFPDHVIDMFINGYRLSLTNHGPTPVKEGSKDPRGGIFDAVFTRGDQSKLLTSRHDFKEKNLKEISDLIKKELTEGKALGLSHTYANVRINHVINLWGADFDSNGNLKAIYVTDSDSNASIGMKKYFVGVNSAGKVAISAKEIKEDNIGAQVLGLFTLSTGQDSWNQTN

SEQ ID NO: 57 - protein, 310 aa, Streptococcus pyogenes
DSFSANQEIRYSEVTPYHVTSVWTKGVTPPANFTQGEDVFHAPYVANQGWYDITKTFNGKDDLLCGAATAGNMLHWWFDQNKDQIKRYLEEHPEKQKINFKGEQMFDVKEAIDTKNHQLDSKLFEYFKEKAFPYLSTKHLGVFPDHVIDMFINGYRLSLTNHGPTPVKRGSKDPRGGIFDAVFTRGNQSKLLTSRHDFKEKNLKEISDLIKKELTEGKALGLSHTYANVRINHVINLWGADFDSNGNLKAIYVTDSDSNASIGMKKYFVGVNSAGKVAISAKEIKEDNIGAQVLGLFTLSTGQDSWNQTN

SEQ ID NO: 58 - protein, 310 aa, Streptococcus pyogenes
DSFSANQEIRYSEVTPYHVTSVWTKGVTPPANFTQGEDVFHAPYVANQGWYDITKTFNGKDDLLCGAATAGNMLHWWFDQNKDQIKRYLEEHPEKQKINFRGEQMFDVKEAIDTKNHQLDSKLFEYFKEKAFPYLSTKHLGVFPDHVIDMFINGYRLSLTNHGPTPVKKGSKDPRGGIFDAVFTRGNQSKLLTSRHDFKEKNLKEISDLIKKELTEGKALGLSHTYANVRINHVINLWGADFDSNGNLKAIYVTDSDSNASIGMKKYFVGVNKAGKVAISAKEIKEDNIGAQVLGLFTLSTGQDSWNQTN

SEQ ID NO: 59 - protein, 310 aa, Streptococcus pyogenes
DSFSANQEIRYSEVTPYHVTSVWTKGVTPPANFTQGEDVFHAPYVANQGWYDITKTFNGKDDLLCGAATAGNMLHWWFDQNKDQIKRYLREHPEKQKINFNGEQMFDVKEAIDTKNHQLDSKLFEYFKEKAFPYLSTKHLGVFPDHVIDMFINGYRLSLTNHGPTPVKEGSKDPRGGIFDAVFTRGNQSKLLTSRHDFKEKNLKEISDLIKKELDEGKALGLSHTYANVRINHVINLWGADFDSNGNLKAIYVTDSDSNASIGMKKYFVGVNSAGKVAISAKEIKEDNIGAQVLGLFTLSTGQDSWNQTN

SEQ ID NO: 60 - protein, 310 aa, Streptococcus pyogenes
DSFSANQEIRYSEVTPYHVTSVWTKGVTPPANFTQGEDVFHAPYVANQGWYDITKTFNGKDDLLCGAATAGNMLHWWFDQNKDQIKRYLKEHPEKQKINFNGEQMFDVKEAIRTKNHQLDSKLFEYFKEKAFPYLSTKHLGVFPDHVIDMFINGYRLSLTNHGPTPVKEGSKDPRGGIFDAVFTRGNQSKLLTSRHDFKEKNLKEISDLIKKELEEGKALGLSHTYANVRINHVINLWGADFDSNGNLKAIYVTDSDSNASIGMKKYFVGVNKAGKVAISAKEIKEDNIGAQVLGLFTLSTGQDSWNQTN

SEQ ID NO: 61 - protein, 310 aa, Streptococcus pyogenes
DSFSANQEIRYSEVTPYHVTSVWTKGVTPPANFTQGEDVFHAPYVANQGWYDITKTFNGKDDLLCGAATAGNMLHWWFDQNKDQIERYLEEHPEKQKINFNGEQMFDVKEAIDTKNHQLDSKLFEYFKEKAFPYLSTKHLGVFPDHVIDMFINGYRLSLTNHGPTPVKEGSKDPRGGIFDAVFTRGNQSKLLTSRHDFKEKNLKEISDLIKEELTKGKALGLSHTYANVRINHVINLWGADFDSNGNLKAIYVTDSDSNASIGMKKYFVGVNSAGKVAISAKEIKEKNIGAQVLGLFTLSTGQKSWNQTN

SEQ ID NO: 62 - protein, 310 aa, Streptococcus pyogenes
DSFSANQEIRYSEVTPYHVTSVWTKGVTPPANFTQGEDVFHAPYVANQGWYDITKTFNGKDDLLCGAATAGNMLHWWFDQNKDQIKRYLKEHPEKQKINFRGEQMFDVKEAIRTKNHQLDSKLFEYFKEKAFPYLSTKHLGVFPDHVIDMFINGYRLSLTNHGPTPVKEGSKDPRGGIFDAVFTRGNQSKLLTSRHDFKEKNLKEISDLIKSELENGKALGLSHTYANVRINHVINLWGADFDSNGNLKAIYVTDSDSNASIGMKKYFVGVNKAGKVAISAKEIKEDNIGAQVLGLFTLSTGQDSWNQTN

SEQ ID NO: 63 - protein, 310 aa, Streptococcus pyogenes
DSFSANQEIRYSEVTPYHVTSVWTKGVTPPANFTQGEDVFHAPYVANQGWYDITKTFNGKDDLLCGAATAGNMLHWWFDQNKDQIKRYLKEHPEKQKINFRGEQMFDVKEAIRTKNHQLDSKLFEYFKEKAFPYLSTKHLGVFPDHVIDMFINGYRLSLTNHGPTPVKKGSKDPRGGIFDAVFTRGNQSKLLTSRHDFKEKNLKEISDLIKKELEEGKALGLSHTYANVRINHVINLWGADFDSNGNLKAIYVTDSDSNASIGMKKYFVGVNSAGKVAISAKEIKEDNIGAQVLGLFTLSTGQDSWNQTN

SEQ ID NO: 64 - protein, 310 aa, Streptococcus pyogenes
DSFSANQEIRYSEVTPYHVTSVWTKGVTPPANFTQGEDVFHAPYVANQGWYDITKTFNGKDDLLCGAATAGNMLHWWFDQNKDQIERYLEEHPEKQKINFRGEQMFDVKEAIDTKNHQLDSKLFEYFKEKAFPYLSTKHLGVFPDHVIDMFINGYRLSLTNHGPTPVKKGSKDPRGGIFDAVFTRGNQSKLLTSRHDFKEKNLKEISDLIKEELTKGKALGLSHTYANVRINHVINLWGADFDSNGNLKAIYVTDSDSNASIGMKKYFVGVNSAGKVAISAKEIKEDNIGAQVLGLFTLSTGQKSWNQTN

SEQ ID NO: 65 - protein, 306 aa, Streptococcus pyogenes
DSFSANQEIRYSEVTPYHVTSVWTKGVTPPANFTQGEDVFHAPYVANQGWYDITKTFNGKDDLLCGAATAGNMLHWWFDQNKDQIKRYLEEHPEKQKINFNGEQMFDVKEAIDTKNHQLDSKLFEYFKEKAFPYLSTKHLGVFPDHVIDMFINGYRLSLTNHGPTPVKEGSKDPRGGIFDAVFTRGDQSKLLTSRHDFKEKNLKEISDLIKKELTEGKALGLSHTYANVRINHVINLWGADFDSNGNLKAIYVTDSDSNASIGMKKYFVGVNSAGKVAISAKEIKEDNIGAQVLGLFTLSTGQDSW

SEQ ID NO: 66 - protein, 290 aa, Streptococcus pyogenes
SVWTKGVTPPANFTQGEDVFHAPYVANQGWYDITKTFNGKDDLLCGAATAGNMLHWWFDQNKDQIKRYLEEHPEKQKINFNGEQMFDVKEAIDTKNHQLDSKLFEYFKEKAFPYLSTKHLGVFPDHVIDMFINGYRLSLTNHGPTPVKEGSKDPRGGIFDAVFTRGDQSKLLTSRHDFKEKNLKEISDLIKKELTEGKALGLSHTYANVRINHVINLWGADFDSNGNLKAIYVTDSDSNASIGMKKYFVGVNSAGKVAISAKEIKEDNIGAQVLGLFTLSTGQDSWNQTN

SEQ ID NO: 67 - protein, 290 aa, Streptococcus pyogenes
SVWTKGVTPPANFTQGEDVFHAPYVANQGWYDITKTFNGKDDLLCGAATAGNMLHWWFDQNKDQIKRYLEEHPEKQKINFKGEQMFDVKEAIDTKNHQLDSKLFEYFKEKAFPYLSTKHLGVFPDHVIDMFINGYRLSLTNHGPTPVKEGSKDPRGGIFDAVFTRGNQSKLLTSRHDFKEKNLKEISDLIKKELTEGKALGLSHTYANVRINHVINLWGADFDSNGNLKAIYVTDSDSNASIGMKKYFVGVNSAGKVAISAKEIKEDNIGAQVLGLFTLSTGQDSWNQTN

SEQ ID NO: 68 - protein, 290 aa, Streptococcus pyogenes
SVWTKGVTPPANFTQGEDVFHAPYVANQGWYDITKTFNGKDDLLCGAATAGNMLHWWFDQNKDQIERYLEEHPEKQKINFKGEQMFDVKKAIDTKNHQLDSKLFEYFKEKAFPYLSTKHLGVFPDHVIDMFINGYRLSLTNHGPTPVKEGSKDPRGGIFDAVFTRGNQSKLLTSRHDFKEKNLKEISDLIKEELTKGKALGLSHTYANVRINHVINLWGADFDSNGNLKAIYVTDSDSNASIGMKKYFVGVNSAGKVAISAKEIKEDNIGAQVLGLFTLSTGQKSWNQTN

SEQ ID NO: 69 - protein, 319 aa, Streptococcus pyogenes
DDYQRNATEAYAKEVPHQITSVWTKGVTPPANFTQGEDVFHAPYVANQGWYDITKTFNGKDDLLCGAATAGNMLHWWFDQNKDQIERYLEEHPEKQKINFKGEQMFDVKKAIDTKNHQLDSKLFEYFKEKAFPYLSTKHLGVFPDHVIDMFINGYRLSLTNHGPTPVKEGSKDPRGGIFDAVFTRGNQSKLLTSRHDFKEKNLKEISDLIKEELTKGKALGLSHTYANVRINHVINLWGADFDSNGNLKAIYVTDSDSNASIGMKKYFVGVNSAGKVAISAKEIKEDNIGAQVLGLFTLSTGQKSWNQTNGGGHHHHHH

SEQ ID NO: 70 - protein, 4 aa, Streptococcus pyogenes
NQTN

SEQ ID NO: 71 - protein, 20 aa, Streptococcus pyogenes
DSFSANQEIRYSEVTPYHVT

SEQ ID NO: 72 - DNA, 963 bp, Streptococcus pyogenes; identical to SEQ ID NO: 33

SEQ ID NO: 73 - DNA, 963 bp, Streptococcus pyogenes
atggatagtttttctgctaatcaagagattagatattcggaagtaacaccttatcacgttacttccgtttggaccaaaggagttactcctccagcaaacttcactcaaggtgaagatgtttttcacgctccttatgttgctaaccaaggatggtatgatattaccaaaacattcaatggaaaagacgatcttctttgcggggctgccacagcagggaatatgcttcactggtggttcgatcaaaacaaagaccaaattaaacgttatttggaagagcatccagaaaagcaaaaaataaacttccgtggcgaacagatgtttgacgtaaaagaagctatcgacactaaaaaccaccagctagatagtaaattatttgaatattttaaagaaaaagctttcccttatctatctactaaacacctaggagttttccctgatcatgtaattgatatgttcattaacggctaccgccttagtctaactaaccacggtccaacgccagtaaaagaaggtagtaaagatccccgaggtggtatttttgacgccgtatttacaagaggtgatcaaagtaagctattgacaagtcgtcatgattttaaagaaaaaaatctcaaagaaatcagtgatctcattaagaaagagttaaccgaaggcaaggctctaggcctatcacacacctacgctaacgtacgcatcaaccatgttataaacctgtggggagctgactttgattctaacgggaaccttaaagctatttatgtaacagactctgatagtaatgcatctattggtatgaagaaatactttgttggtgttaattccgctggaaaagtagctatttctgctaaagaaataaaagaagataatataggtgctcaagtactagggttatttacactttcaacagggcaagatagttggaatcagaccaatggcggtggccatcatcaccatcaccactaa

SEQ ID NO: 74 - DNA, 963 bp, Streptococcus pyogenes
atggatagtttttctgctaatcaagagattagatattcggaagtaacaccttatcacgttacttccgtttggaccaaaggagttactcctccagcaaacttcactcaaggtgaagatgtttttcacgctccttatgttgctaaccaaggatggtatgatattaccaaaacattcaatggaaaagacgatcttctttgcggggctgccacagcagggaatatgcttcactggtggttcgatcaaaacaaagaccaaattaaacgttatttggaagagcatccagaaaagcaaaaaataaacttcaaaggcgaacagatgtttgacgtaaaagaagctatcgacactaaaaaccaccagctagatagtaaattatttgaatattttaaagaaaaagctttcccttatctatctactaaacacctaggagttttccctgatcatgtaattgatatgttcattaacggctaccgccttagtctaactaaccacggtccaacgccagtaaaacgtggtagtaaagatccccgaggtggtatttttgacgccgtatttacaagaggtaaccaaagtaagctattgacaagtcgtcatgattttaaagaaaaaaatctcaaagaaatcagtgatctcattaagaaagagttaaccgaaggcaaggctctaggcctatcacacacctacgctaacgtacgcatcaaccatgttataaacctgtggggagctgactttgattctaacgggaaccttaaagctatttatgtaacagactctgatagtaatgcatctattggtatgaagaaatactttgttggtgttaattccgctggaaaagtagctatttctgctaaagaaataaaagaagataatataggtgctcaagtactagggttatttacactttcaacagggcaagatagttggaatcagaccaatggcggtggccatcatcaccatcaccactaa

SEQ ID NO: 75 - DNA, 963 bp, Streptococcus pyogenes
atggatagtttttctgctaatcaagagattagatattcggaagtaacaccttatcacgttacttccgtttggaccaaaggagttactcctccagcaaacttcactcaaggtgaagatgtttttcacgctccttatgttgctaaccaaggatggtatgatattaccaaaacattcaatggaaaagacgatcttctttgcggggctgccacagcagggaatatgcttcactggtggttcgatcaaaacaaagaccaaattaaacgttatttggaagagcatccagaaaagcaaaaaataaacttccgtggcgaacagatgtttgacgtaaaagaagctatcgacactaaaaaccaccagctagatagtaaattatttgaatattttaaagaaaaagctttcccttatctatctactaaacacctaggagttttccctgatcatgtaattgatatgttcattaacggctaccgccttagtctaactaaccacggtccaacgccagtaaaaaaaggtagtaaagatccccgaggtggtatttttgacgccgtatttacaagaggtaaccaaagtaagctattgacaagtcgtcatgattttaaagaaaaaaatctcaaagaaatcagtgatctcattaagaaagagttaaccgaaggcaaggctctaggcctatcacacacctacgctaacgtacgcatcaaccatgttataaacctgtggggagctgactttgattctaacgggaaccttaaagctatttatgtaacagactctgatagtaatgcatctattggtatgaagaaatactttgttggtgttaataaagctggaaaagtagctatttctgctaaagaaataaaagaagataatataggtgctcaagtactagggttatttacactttcaacagggcaagatagttggaatcagaccaatggcggtggccatcatcaccatcaccactaa

SEQ ID NO: 76 - DNA, 963 bp, Streptococcus pyogenes
atggatagtttttctgctaatcaagagattagatattcggaagtaacaccttatcacgttacttccgtttggaccaaaggagttactcctccagcaaacttcactcaaggtgaagatgtttttcacgctccttatgttgctaaccaaggatggtatgatattaccaaaacattcaatggaaaagacgatcttctttgcggggctgccacagcagggaatatgcttcactggtggttcgatcaaaacaaagaccaaattaaacgttatttgcgtgagcatccagaaaagcaaaaaataaacttcaatggcgaacagatgtttgacgtaaaagaagctatcgacactaaaaaccaccagctagatagtaaattatttgaatattttaaagaaaaagctttcccttatctatctactaaacacctaggagttttccctgatcatgtaattgatatgttcattaacggctaccgccttagtctaactaaccacggtccaacgccagtaaaagaaggtagtaaagatccccgaggtggtatttttgacgccgtatttacaagaggtaaccaaagtaagctattgacaagtcgtcatgattttaaagaaaaaaatctcaaagaaatcagtgatctcattaagaaagagttagatgaaggcaaggctctaggcctatcacacacctacgctaacgtacgcatcaaccatgttataaacctgtggggagctgactttgattctaacgggaaccttaaagctatttatgtaacagactctgatagtaatgcatctattggtatgaagaaatactttgttggtgttaattccgctggaaaagtagctatttctgctaaagaaataaaagaagataatataggtgctcaagtactagggttatttacactttcaacagggcaagatagttggaatcagaccaatggcggtggccatcatcaccatcaccactaa

SEQ ID NO: 77 - DNA, 963 bp, Streptococcus pyogenes
atggatagtttttctgctaatcaagagattagatattcggaagtaacaccttatcacgttacttccgtttggaccaaaggagttactcctccagcaaacttcactcaaggtgaagatgtttttcacgctccttatgttgctaaccaaggatggtatgatattaccaaaacattcaatggaaaagacgatcttctttgcggggctgccacagcagggaatatgcttcactggtggttcgatcaaaacaaagaccaaattaaacgttatttgaaagagcatccagaaaagcaaaaaataaacttcaatggcgaacagatgtttgacgtaaaagaagctatccgtactaaaaaccaccagctagatagtaaattatttgaatattttaaagaaaaagctttcccttatctatctactaaacacctaggagttttccctgatcatgtaattgatatgttcattaacggctaccgccttagtctaactaaccacggtccaacgccagtaaaagaaggtagtaaagatccccgaggtggtatttttgacgccgtatttacaagaggtaaccaaagtaagctattgacaagtcgtcatgattttaaagaaaaaaatctcaaagaaatcagtgatctcattaagaaagagttagaagaaggcaaggctctaggcctatcacacacctacgctaacgtacgcatcaaccatgttataaacctgtggggagctgactttgattctaacgggaaccttaaagctatttatgtaacagactctgatagtaatgcatctattggtatgaagaaatactttgttggtgttaataaagctggaaaagtagctatttctgctaaagaaataaaagaagataatataggtgctcaagtactagggttatttacactttcaacagggcaagatagttggaatcagaccaatggcggtggccatcatcaccatcaccactaa

SEQ ID NO: 78 - DNA, 963 bp, Streptococcus pyogenes
atggatagtttttctgctaatcaagagattagatattcggaagtaacaccttatcacgttacttccgtttggaccaaaggagttactcctccagcaaacttcactcaaggtgaagatgtttttcacgctccttatgttgctaaccaaggatggtatgatattaccaaaacattcaatggaaaagacgatcttctttgcggggctgccacagcagggaatatgcttcactggtggttcgatcaaaacaaagaccaaattgaacgttatttggaagagcatccagaaaagcaaaaaataaacttcaatggcgaacagatgtttgacgtaaaagaagctatcgacactaaaaaccaccagctagatagtaaattatttgaatattttaaagaaaaagctttcccttatctatctactaaacacctaggagttttccctgatcatgtaattgatatgttcattaacggctaccgccttagtctaactaaccacggtccaacgccagtaaaagaaggtagtaaagatccccgaggtggtatttttgacgccgtatttacaagaggtaaccaaagtaagctattgacaagtcgtcatgattttaaagaaaaaaatctcaaagaaatcagtgatctcattaaggaagagttaaccaaaggcaaggctctaggcctatcacacacctacgctaacgtacgcatcaaccatgttataaacctgtggggagctgactttgattctaacgggaaccttaaagctatttatgtaacagactctgatagtaatgcatctattggtatgaagaaatactttgttggtgttaattccgctggaaaagtagctatttctgctaaagaaataaaagaaaaaaatataggtgctcaagtactagggttatttacactttcaacagggcaaaaaagttggaatcagaccaatggcggtggccatcatcaccatcaccactaa

SEQ ID NO: 79 - DNA, 963 bp, Streptococcus pyogenes
atggatagtttttctgctaatcaagagattagatattcggaagtaacaccttatcacgttacttccgtttggaccaaaggagttactcctccagcaaacttcactcaaggtgaagatgtttttcacgctccttatgttgctaaccaaggatggtatgatattaccaaaacattcaatggaaaagacgatcttctttgcggggctgccacagcagggaatatgcttcactggtggttcgatcaaaacaaagaccaaattaaacgttatttgaaagagcatccagaaaagcaaaaaataaacttccgtggcgaacagatgtttgacgtaaaagaagctatccgtactaaaaaccaccagctagatagtaaattatttgaatattttaaagaaaaagctttcccttatctatctactaaacacctaggagttttccctgatcatgtaattgatatgttcattaacggctaccgccttagtctaactaaccacggtccaacgccagtaaaagaaggtagtaaagatccccgaggtggtatttttgacgccgtatttacaagaggtaaccaaagtaagctattgacaagtcgtcatgattttaaagaaaaaaatctcaaagaaatcagtgatctcattaagagtgagttagaaaacggcaaggctctaggcctatcacacacctacgctaacgtacgcatcaaccatgttataaacctgtggggagctgactttgattctaacgggaaccttaaagctatttatgtaacagactctgatagtaatgcatctattggtatgaagaaatactttgttggtgttaataaagctggaaaagtagctatttctgctaaagaaataaaagaagataatataggtgctcaagtactagggttatttacactttcaacagggcaagatagttggaatcagaccaatggcggtggccatcatcaccatcaccactaa

SEQ ID NO: 80 - DNA, 963 bp, Streptococcus pyogenes
atggatagtttttctgctaatcaagagattagatattcggaagtaacaccttatcacgttacttccgtttggaccaaaggagttactcctccagcaaacttcactcaaggtgaagatgtttttcacgctccttatgttgctaaccaaggatggtatgatattaccaaaacattcaatggaaaagacgatcttctttgcggggctgccacagcagggaatatgcttcactggtggttcgatcaaaacaaagaccaaattaaacgttatttgaaagagcatccagaaaagcaaaaaataaacttccgtggcgaacagatgtttgacgtaaaagaagctatccgtactaaaaaccaccagctagatagtaaattatttgaatattttaaagaaaaagctttcccttatctatctactaaacacctaggagttttccctgatcatgtaattgatatgttcattaacggctaccgccttagtctaactaaccacggtccaacgccagtaaaaaaaggtagtaaagatccccgaggtggtatttttgacgccgtatttacaagaggtaaccaaagtaagctattgacaagtcgtcatgattttaaagaaaaaaatctcaaagaaatcagtgatctcattaagaaagagttagaagaaggcaaggctctaggcctatcacacacctacgctaacgtacgcatcaaccatgttataaacctgtggggagctgactttgattctaacgggaaccttaaagctatttatgtaacagactctgatagtaatgcatctattggtatgaagaaatactttgttggtgttaattccgctggaaaagtagctatttctgctaaagaaataaaagaagataatataggtgctcaagtactagggttatttacactttcaacagggcaagatagttggaatcagaccaatggcggtggccatcatcaccatcaccactaa

SEQ ID NO: 81 - DNA, 963 bp, Streptococcus pyogenes
atggatagtttttctgctaatcaagagattagatattcggaagtaacaccttatcacgttacttccgtttggaccaaaggagttactcctccagcaaacttcactcaaggtgaagatgtttttcacgctccttatgttgctaaccaaggatggtatgatattaccaaaacattcaatggaaaagacgatcttctttgcggggctgccacagcagggaatatgcttcactggtggttcgatcaaaacaaagaccaaattgaacgttatttggaagagcatccagaaaagcaaaaaataaacttccgtggcgaacagatgtttgacgtaaaagaagctatcgacactaaaaaccaccagctagatagtaaattatttgaatattttaaagaaaaagctttcccttatctatctactaaacacctaggagttttccctgatcatgtaattgatatgttcattaacggctaccgccttagtctaactaaccacggtccaacgccagtaaaaaaaggtagtaaagatccccgaggtggtatttttgacgccgtatttacaagaggtaaccaaagtaagctattgacaagtcgtcatgattttaaagaaaaaaatctcaaagaaatcagtgatctcattaaggaagagttaaccaaaggcaaggctctaggcctatcacacacctacgctaacgtacgcatcaaccatgttataaacctgtggggagctgactttgattctaacgggaaccttaaagctatttatgtaacagactctgatagtaatgcatctattggtatgaagaaatactttgttggtgttaattccgctggaaaagtagctatttctgctaaagaaataaaagaagataatataggtgctcaagtactagggttatttacactttcaacagggcaaaaaagttggaatcagaccaatggcggtggccatcatcaccatcaccactaa

SEQ ID NO: 82 - DNA, 957 bp, Streptococcus pyogenes
atggatagtttttctgctaatcaagagattagatattcggaagtaacaccttatcacgttacttccgtttggaccaaaggagttactcctccagcaaacttcactcaaggtgaagatgtttttcacgctccttatgttgctaaccaaggatggtatgatattaccaaaacattcaatggaaaagacgatcttctttgcggggctgccacagcagggaatatgcttcactggtggttcgatcaaaacaaagaccaaattaaacgttatttggaagagcatccagaaaagcaaaaaataaacttcaatggcgaacagatgtttgacgtaaaagaagctatcgacactaaaaaccaccagctagatagtaaattatttgaatattttaaagaaaaagctttcccttatctatctactaaacacctaggagttttccctgatcatgtaattgatatgttcattaacggctaccgccttagtctaactaaccacggtccaacgccagtaaaagaaggtagtaaagatccccgaggtggtatttttgacgccgtatttacaagaggtgatcaaagtaagctattgacaagtcgtcatgattttaaagaaaaaaatctcaaagaaatcagtgatctcattaagaaagagttaaccgaaggcaaggctctaggcctatcacacacctacgctaacgtacgcatcaaccatgttataaacctgtggggagctgactttgattctaacgggaaccttaaagctatttatgtaacagactctgatagtaatgcatctattggtatgaagaaatactttgttggtgttaattccgctggaaaagtagctatttctgctaaagaaataaaagaagataatataggtgctcaagtactagggttatttacactttcaacagggcaagatagttggggtggcggcggtggccatcatcaccatcaccactaa

SEQ ID NO: 83 - DNA, 903 bp, Streptococcus pyogenes
atgtccgtttggaccaaaggagttactcctccagcaaacttcactcaaggtgaagatgtttttcacgctccttatgttgctaaccaaggatggtatgatattaccaaaacattcaatggaaaagacgatcttctttgcggggctgccacagcagggaatatgcttcactggtggttcgatcaaaacaaagaccaaattaaacgttatttggaagagcatccagaaaagcaaaaaataaacttcaatggcgaacagatgtttgacgtaaaagaagctatcgacactaaaaaccaccagctagatagtaaattatttgaatattttaaagaaaaagctttcccttatctatctactaaacacctaggagttttccctgatcatgtaattgatatgttcattaacggctaccgccttagtctaactaaccacggtccaacgccagtaaaagaaggtagtaaagatccccgaggtggtatttttgacgccgtatttacaagaggtgatcaaagtaagctattgacaagtcgtcatgattttaaagaaaaaaatctcaaagaaatcagtgatctcattaagaaagagttaaccgaaggcaaggctctaggcctatcacacacctacgctaacgtacgcatcaaccatgttataaacctgtggggagctgactttgattctaacgggaaccttaaagctatttatgtaacagactctgatagtaatgcatctattggtatgaagaaatactttgttggtgttaattccgctggaaaagtagctatttctgctaaagaaataaaagaagataatataggtgctcaagtactagggttatttacactttcaacagggcaagatagttggaatcagaccaatggcggtggccatcatcaccatcaccactaa

SEQ ID NO: 84 - DNA, 903 bp, Streptococcus pyogenes
atgtccgtttggaccaaaggagttactcctccagcaaacttcactcaaggtgaagatgtttttcacgctccttatgttgctaaccaaggatggtatgatattaccaaaacattcaatggaaaagacgatcttctttgcggggctgccacagcagggaatatgcttcactggtggttcgatcaaaacaaagaccaaattaaacgttatttggaagagcatccagaaaagcaaaaaataaacttcaaaggcgaacagatgtttgacgtaaaagaagctatcgacactaaaaaccaccagctagatagtaaattatttgaatattttaaagaaaaagctttcccttatctatctactaaacacctaggagttttccctgatcatgtaattgatatgttcattaacggctaccgccttagtctaactaaccacggtccaacgccagtaaaagaaggtagtaaagatccccgaggtggtatttttgacgccgtatttacaagaggtaaccaaagtaagctattgacaagtcgtcatgattttaaagaaaaaaatctcaaagaaatcagtgatctcattaagaaagagttaaccgaaggcaaggctctaggcctatcacacacctacgctaacgtacgcatcaaccatgttataaacctgtggggagctgactttgattctaacgggaaccttaaagctatttatgtaacagactctgatagtaatgcatctattggtatgaagaaatactttgttggtgttaattccgctggaaaagtagctatttctgctaaagaaataaaagaagataatataggtgctcaagtactagggttatttacactttcaacagggcaagatagttggaatcagaccaatggcggtggccatcatcaccatcaccactaa

SEQ ID NO: 85 - DNA, 903 bp, Streptococcus pyogenes
atgtccgtttggaccaaaggagttactcctccagcaaacttcactcaaggtgaagatgtttttcacgctccttatgttgctaaccaaggatggtatgatattaccaaaacattcaatggaaaagacgatcttctttgcggggctgccacagcagggaatatgcttcactggtggttcgatcaaaacaaagaccaaattgaacgttatttggaagagcatccagaaaagcaaaaaataaacttcaaaggcgaacagatgtttgacgtaaaaaaagctatcgacactaaaaaccaccagctagatagtaaattatttgaatattttaaagaaaaagctttcccttatctatctactaaacacctaggagttttccctgatcatgtaattgatatgttcattaacggctaccgccttagtctaactaaccacggtccaacgccagtaaaagaaggtagtaaagatccccgaggtggtatttttgacgccgtatttacaagaggtaaccaaagtaagctattgacaagtcgtcatgattttaaagaaaaaaatctcaaagaaatcagtgatctcattaaggaagagttaaccaaaggcaaggctctaggcctatcacacacctacgctaacgtacgcatcaaccatgttataaacctgtggggagctgactttgattctaacgggaaccttaaagctatttatgtaacagactctgatagtaatgcatctattggtatgaagaaatactttgttggtgttaattccgctggaaaagtagctatttctgctaaagaaataaaagaagataatataggtgctcaagtactagggttatttacactttcaacagggcaaaaaagttggaatcagaccaatggcggtggccatcatcaccatcaccactaa

SEQ ID NO: 86 - DNA, 963 bp, Streptococcus pyogenes
atggacgattaccaaaggaatgctacggaagcttatgccaaagaagtaccacatcagatcacttccgtttggaccaaaggagttactcctccagcaaacttcactcaaggtgaagatgtttttcacgctccttatgttgctaaccaaggatggtatgatattaccaaaacattcaatggaaaagacgatcttctttgcggggctgccacagcagggaatatgcttcactggtggttcgatcaaaacaaagaccaaattgaacgttatttggaagagcatccagaaaagcaaaaaataaacttcaaaggcgaacagatgtttgacgtaaaaaaagctatcgacactaaaaaccaccagctagatagtaaattatttgaatattttaaagaaaaagctttcccttatctatctactaaacacctaggagttttccctgatcatgtaattgatatgttcattaacggctaccgccttagtctaactaaccacggtccaacgccagtaaaagaaggtagtaaagatccccgaggtggtatttttgacgccgtatttacaagaggtaaccaaagtaagctattgacaagtcgtcatgattttaaagaaaaaaatctcaaagaaatcagtgatctcattaaggaagagttaaccaaaggcaaggctctaggcctatcacacacctacgctaacgtacgcatcaaccatgttataaacctgtggggagctgactttgattctaacgggaaccttaaagctatttatgtaacagactctgatagtaatgcatctattggtatgaagaaatactttgttggtgttaattccgctggaaaagtagctatttctgctaaagaaataaaagaagataatataggtgctcaagtactagggttatttacactttcaacagggcaaaaaagttggaatcagaccaatggcggtggccatcatcaccatcaccactaa

SEQ ID NO: 87 - protein, 19 aa, Streptococcus pyogenes
SFSANQEIRYSEVTPYHVT

SEQ ID NO: 88 - protein, 19 aa, Streptococcus pyogenes
DYQRNATEAYAKEVPHQIT

SEQ ID NO: 89 - protein, 20 aa, Streptococcus pyogenes
DDYQRNATEAYAKEVPHQIT

SEQ ID NO: 90 - protein, 959 aa, Streptococcus pyogenes
EEKTVQVQKGLPSIDSLHYLSENSKKEFKEELSKAGQESQKVKEILAKAQQADKQAQELAKMKIPEKIPMKPLHGPLYGGYFRTWHDKTSDPTEKDKVNSMGELPKEVDLAFIFHDWTKDYSLFWKELATKHVPKLNKQGTRVIRTIPWRFLAGGDNSGIAEDTSKYPNTPEGNKALAKAIVDEYVYKYNLDGLDVDVEHDSIPKVDKKEDTAGVERSIQVFEEIGKLIGPKGVDKSRLFIMDSTYMADKNPLIERGAPYINLLLVQVYGSQGEKGGWEPVSNRPEKTMEERWQGYSKYIRPEQYMIGFSFYEENAQEGNLWYDINSRKDEDKANGINTDITGTRAERYARWQPKTGGVKGGIFSYAIDRDGVAHQPKKYAKQKEFKDATDNIFHSDYSVSKALKTVMLKDKSYDLIDEKDFPDKALREAVMAQVGTRKGDLERFNGTLRLDNPAIQSLEGLNKFKKLAQLDLIGLSRITKLDRSVLPANMKPGKDTLETVLETYKKDNKEEPATIPPVSLKVSGLTGLKELDLSGFDRETLAGLDAATLTSLEKVDISGNKLDLAPGTENRQIFDTMLSTISNHVGSNEQTVKFDKQKPTGHYPDTYGKTSLRLPVANEKVDLQSQLLFGTVTNQGTLINSEADYKAYQNHKIAGRSFVDSNYHYNNFKVSYENYTVKVTDSTLGTTTDKTLATDKEETYKVDFFSPADKTKAVHTAKVIVGDEKTMMVNLAEGATVIGGSADPVNARKVFDGQLGSETDNISLGWDSKQSIIFKLKEDGLIKHWRFFNDSARNPETTNKPIQEASLQIFNIKDYNLDNLLENPNKFDDEKYWITVDTYSAQGERATAFSNTLNNITSKYWRVVFDTKGDRYSSPVVPELQILGYPLPNADTIMKTVTTAKELSQQKDKFSQKMLDELKIKEMALETSLNSKIFDVTAINANAGVLKDCIEKRQLLKK